European Patent Application EP 4 428 226 A1, published September 11, 2024. Title: RECOMBINANT MICROORGANISM CONSTRUCTED BASED ON LYSINE EFFLUX PROTEIN AND METHOD FOR PRODUCING LYSINE. Applicant: Tianjin Institute of Industrial Biotechnology, Chinese Academy of Sciences. The sequence listing filed with the application follows.

SEQUENCE LISTING (25 sequences)

SEQ ID NO: 1 - protein, 299 aa, Brenneria salicis
MYSGLLIILLPLLFGYLLPLRAKKVLQTINQLLSWMVYVILFLMGISLAFLDNLGSNLLLIFRYAAVFFVCIIAANALSLWLWGKRDVWPGKFPQEAPPSRLYMILDSLKLCLVVFGGFLLGLTQWPGLIHASEGSEYALILLLFFVGIQLRNSGMTLRQIVLNRRGMSIALVVGVSALAGGLLAARVLSLPLKTGLAIASGYGWYSLSGILLTDALGPVIGSAAFFNDLARELLAIMLIPALTRRNRACALGLCGATSMDFTLLVLQRSAGVDMVPAAIVHGFLLSLVAPVFMALFSS

SEQ ID NO: 2 - protein, 309 aa, Halomonas gudaonensis
MLSGLLLVLLPLLLGYLVPVHHTGAMDVINRSVNAAIYVILLLMGVGLAGLDDLASQLSRMGSQALLLFLLLSACNLAALAWLARRLRMRIEPGRSVADAPTSKLAALAGSLALVGVVIGGVLTGLVASGLSAGEGFFSGAETLAEGVLYLLLALIGCQLRNSGMPLRQILLNRRGLAIAATLAASSLVGGLVAAPLLSLAWNEGLALAAGFGWYSLSGILIGDGLGAQMGGVAFFNDLLRELAAFVLIPLTIRRHAPLAIGYGGATAMDFTLPVIQQHGGVACVPVAVVSGFLLSLLSPPLILFFLSL

SEQ ID NO: 3 - protein, 300 aa, Ferrimonas sediminum
MSLESLVILLPLFAGYLIPVTRPALLTGIDKLLSAIVYLILALMGLSLAQVDNLAGELSSILQLVALLIGLSLVLNLALLPLVDRRWPMALTLNNGHQPLGKMMLESLKLAAVVVGGVALGLVLPVGHQAIESGANAALMLLLGLIGIQLRASNLGLRAILLNPRGLAIAAIVAVTSLLAGALTALIAGLPVIHGITLAAGFGWYSLSGILITDGLGPVMGSVAFLFDLSRELIAIVIIPMLMRRSPASAIGYGGATAMDFTLPVLQQTGGAPVVPVAIVSGFLLSLASPVLIPFLLSLA

SEQ ID NO: 4 - protein, 302 aa, unclassified Marinobacter
MLASALLILVPLFVGFAFHVENRRVLSTINHSLEALVYLILALLGISLGQLEGLAEQLNRMTGQVLVLVFGLLIANVAGLWLWHRWQPMTLAAAEDSQGNVGYRRLFLGAAKPLLAVIAGMALGHWLLPAVSWIEDVASGALMLLLLLIGLQLRNAGLSLRRLLMNRQGLGIAVTLALTSLLAGLAIAPFYDLPLMHVLALTSGFGWYSLSGIVVGDALGPAWGGVAFLNDVLREIIALVLIPLIIARRPAMAIGYGGATAMDFTLPIIRRSGGLETVPVAIASGFILSFLSPVLMGLFLAG

SEQ ID NO: 5 - protein, 305 aa, Kerstersia gyiorum
MTALSSLMPIVGALAGGWAASHVLPRTLRHWLIRLIGPLVWLLLFLIGMEFGAVLSSAEALGSALYTAGVLALFTTLVPCLLIWLLIRRTRGSATAPRREANTATFWQPVKECGIALSMVVLGGLAFTWMPASIAHAHPLPSSWTLLLVLIVLVGIDLGQVDLKGRLWSFKAFAIPLLVVLGSLLGACAAAWATGENLQVALALASGFGWFSLSSVMIGEALGQNYGTIALMTDLLRELLAIVILYMAGMHYPLPAVGSAGATALDTTLPIVKQTCAPDIVPLALVSGFILTVLAPFMIMVFLAH

SEQ ID NO: 6 - protein, 304 aa, Pseudomonas viridiflava
MNNALWATVPILLALVLGFGLGQYVNDQYRNYVSRCVGILVWVLLFSLGAEFGSVLGNPQLAARSLFVGITFAMTCTLATWLLIHLLTATSDRKAAFRLTELLSSLVEGLKSCTVTLSIVTLGAIYAHFPIDWITSIWKPTLGDMICVLVFLVGIELAKLNLGRDLFTPRSITVPLITVVGTLSGGLLAAWIVDEPLKIGLVLASGFGWMSLSSAMVSETLGKSYGSMVLIADLLRELLAITLLYIFGMKAPLACIGATGVTSLDSTLPIVRVTCPEEVIPYAVVSGLILTVVSPLFIAFFLTL

SEQ ID NO: 7 - DNA, 900 bp, Brenneria salicis
  source 1..900: mol_type = other DNA
atgtattcgggattattaattattttattgccattactgtttggctatctgttgcctttgcgcgcgaaaaaagtcctacagacaattaatcagctattgagttggatggtgtacgtcattctatttttaatgggaattagcctggcttttctggataacctcggcagcaatctgttactgatttttcgttacgccgccgttttctttgtgtgcatcattgccgccaatgccttgtcgctatggctgtggggaaaacgtgatgtctggccgggaaaatttccccaggaagcgccgccttcccgcctgtatatgattctggattcgttaaagctctgtctggtggtatttggcggttttctgctggggttgacgcaatggcctggtttgatccatgccagtgaaggcagcgaatacgcgctgattctgttgttgtttttcgtcggaatacagttacgcaacagcggaatgacgctacgtcaaatcgtgttgaatcgacggggaatgtcgattgcgttggttgtcggcgtcagtgcgctggcaggcggtttactcgccgccagggtgctcagcctgccgctcaaaaccgggctggcgatagcatccggctatggctggtattcgttatccggcattctgctgaccgacgccttaggcccggtgatcggcagcgcggcctttttcaacgatctggcgcgagaactgttagccatcatgttgattcccgcgctgacacgacgcaaccgcgcctgtgcgctcggactgtgcggcgcgacgtcgatggatttcacgttgctggtgttgcaacgcagcgccggggtcgatatggtgccggcggccattgtgcacggttttctattgagtcttgtcgcgccggtattcatggcgctattttcctcctga

SEQ ID NO: 8 - DNA, 930 bp, Halomonas gudaonensis
  source 1..930: mol_type = other DNA
atgctgagcggtctgctgctcgtcctgctgccgttgctgctgggctatctggtgccggtgcatcacaccggcgcaatggatgtcatcaaccgcagcgtcaacgccgccatctacgtgatcctgctgttgatgggtgtgggcctggccggcctcgacgacctggccagccagctctcgcgcatgggcagccaggcactgctgctgttcttgctgctctccgcctgcaacctggcggcattggcctggctggcccgacgcctgcggatgcgcatcgaacccggccgctcggtggccgacgcgccgaccagcaagctcgcggccctggccggctcgctggcactggtgggggtggtgatcggcggcgtgctgacggggctggtcgccagcggcctgagtgcgggtgaagggtttttcagcggtgccgaaacgctggccgaaggtgtgctctacctgctgttggcgctgatcggctgccagctgcgcaactccggcatgccactgcgccagattctgctcaaccgccgcggcctggccattgccgccaccctggcggccagttcgctggtgggtgggctggttgccgcgccactgctctccctcgcctggaacgaagggctggcgctggctgccggcttcggctggtactcgctttccggcatcctgatcggcgacgggctgggcgcccagatgggcggcgtggccttcttcaacgacctgctgcgcgaactggcagccttcgtgctgatcccgctgaccatccgccgccacgccccgctggccatcggctacggcggcgccacggccatggatttcaccctgccagtgattcagcagcacggtggcgtggcttgcgtacccgtcgccgtggtctcgggctttctgctctcgctgctatcgccgccgttgatcctgtttttcctgtcattgtga

SEQ ID NO: 9 - DNA, 903 bp, Ferrimonas sediminum
  source 1..903: mol_type = other DNA
atgtccctagaatccctggttattcttctccccctgtttgccggttacctgattccggtaacccgcccggccctgctgaccggcatcgacaagctgctgagcgccatcgtctatctgattctggcgttgatggggctgtcactggcccaggtggacaacctggccggcgagctgagcagcatcctgcagttagtggcgctgctgatcggtttgagcctggtactgaacctggcgctgttgccgctggtggatcgacgctggcccatggctctgaccctgaacaacggccatcagccactgggcaagatgatgttggaatcgttgaaactggcggccgtggtggttggcggggtggcgttggggctggtgctacccgtcggccatcaggccattgagtctggcgccaacgccgcgctgatgctgctgttggggctgatcgggattcagctgcgggcgtccaacctggggctacgggcgattctgctcaaccccaggggactggccatcgccgccattgtcgccgtcacctcactgctggccggcgccctgaccgccctgatcgccgggctgccggtgattcacggcatcaccctggcggcgggctttggctggtactccctcagcggcatcctgatcaccgacggcctggggccggtaatgggctcggtggccttcctgttcgacctcagccgcgagctgatcgccattgtgattattccgatgctgatgcgccgctcgccggcgtccgccatcggctacggcggcgccacggccatggacttcaccctgccggtactgcagcagaccggcggtgccccggtggtgccagtggccattgtgtccggcttcctgctgagcctggccagcccggtgctgatccccttcctgctgtcgctggcgtaa

SEQ ID NO: 10 - DNA, 909 bp, unclassified Marinobacter
  source 1..909: mol_type = other DNA
atgcttgccagcgcgctgctgatcctggtgcctctctttgtcggttttgccttccacgtcgagaatcgccgtgtactgtcaacgatcaaccattcgctggaagcgttggtgtatctcattctggctctgctcggcatcagcctgggccagcttgagggattggcggagcaattgaaccggatgaccggtcaggtgctggtcctggttttcggattgctgatcgccaacgttgccggcctctggttgtggcatcgctggcagccaatgacgctggcagcggccgaggacagtcagggcaatgtgggttaccggcgtttgttcctcggtgcggcaaaaccactgctggcggtgattgccggcatggcgctgggccactggctgttgcccgcagtgagctggatcgaggacgtggccagcggggcgctgatgctcctgctgctgctgatcggcctgcagttgcgtaatgccggtctgtccctgcggcgcctgctgatgaaccggcagggtctggggattgctgtcaccctggcgctgacctcgctgctggcgggcctggcgatcgcgccgttttatgatctgcccctgatgcatgtgttggcgctgacgtcgggctttggctggtattccctgtcgggcatcgtggtgggggatgcgttggggccggcctggggcggcgtggcgtttctcaacgatgtcctgcgggaaatcatcgccctggtgctgattccattgatcatcgcccggcggccagccatggccatcggctacggcggcgccaccgccatggacttcaccctgccgatcatccgccgcagcggcggcctggaaaccgtgcccgtcgcgatcgcctcgggtttcatcctgtccttcctgtcgcccgttctgatgggcctcttcctcgccggctga

SEQ ID NO: 11 - DNA, 918 bp, Kerstersia gyiorum
  source 1..918: mol_type = other DNA
atgaccgccctctcctctctgatgccgattgtcggcgcgctcgccggcggctgggccgccagccatgtcttgccgcgcacgctgcggcactggctgatacggttgatcggcccgctggtctggctgctgctgtttctgatcggcatggaattcggcgccgtgctctcgtcggccgaagcgctgggcagcgcgctctacacagccggcgtactggccttgttcaccaccctggtgccatgcctgctgatctggctgctgatacggcgcacccgaggcagcgcaacggcgccgcgccgcgaagccaataccgccacgttctggcaaccagtgaaagaatgcggcattgccttgtccatggtggtgctcggggggctggcctttacctggatgcccgccagcattgcgcacgcccatccgttgccatcgagctggacgctgctgttggttctgatcgtactggtcggcatcgacctgggccaggtcgacctgaaaggccggctttggtcattcaaggccttcgccatcccgctgctggtcgtgctcggctcgttgctgggcgcctgcgctgccgcctgggcgaccggtgaaaatcttcaggtcgcgcttgcgctggcgtcgggcttcggctggttttcgctgtccagcgtcatgattggcgaggccctgggccagaactacggcaccatcgccctgatgaccgacttgctgcgtgagctgctggccattgtcatcctctatatggccggcatgcattatccgctgcccgccgtcggcagcgcgggcgctaccgccctggacaccaccttgcccatcgtcaagcagacctgcgcgccggatattgttcccctggcactggtgagcggtttcatcctgaccgtgcttgcgcccttcatgatcatggtgttcctggcgcactga

SEQ ID NO: 12 - DNA, 915 bp, Pseudomonas viridiflava
  source 1..915: mol_type = other DNA
atgaacaacgcactatgggcgactgtgcctattcttttggcacttgtccttgggtttgggctcggccaatacgtaaacgatcagtatcgaaactacgtctcacgatgcgtcgggatactggtctgggtgctacttttttcgctgggtgcagagtttggtagcgtgctcggcaatccgcagttggcagcaagatctctgtttgtcggcatcacctttgccatgacctgtacccttgccacttggctgttgattcatttgttgacagctacgagtgatcgcaaagctgccttcaggctgacggaactgctcagttctcttgtcgaaggtttgaagagttgcaccgtcactttgtccatcgtcacgttgggagcaatctatgctcatttcccaattgactggatcacctcaatctggaagcccacgctgggtgacatgatttgcgtgctggtttttctagtgggtattgagctggctaagttgaatttgggccgcgatctcttcactcccagatccatcaccgttcccctcatcacggtagtgggtacattatccggcggacttctggctgcctggatagtcgatgaaccactcaagatcggactggtgcttgcttcggggtttggctggatgagcttgtccagtgcaatggtcagcgaaacactgggcaaatcctacggctcgatggttttgattgcggacctcctgcgagaactcctggctatcaccctgctttacattttcggcatgaaagcgcctctggcctgcattggcgccactggcgtcacttcgctggactcaaccttgccgattgttcgcgtgacatgccccgaagaagtcattccctacgctgttgtcagcggcctgattctgacagtggtttcccctctgtttatcgcttttttcctgacgctatga

SEQ ID NO: 13 - protein, 250 aa, synthetic construct
  REGION 1..250: note = GntR1 with R102A mutation
MTPANESPMTNPLGSAPTPAKPLLDSVLDELGQDIISGKVAVGDTFKLMDIGERFGISRTVAREAMRALEQLGLVASSRRIGITVLPQEEWAVFDKSIIRWALNDEGQREGQLQSLTELRIAIEPIAARSVALHASTAELEKIRALATEMRQLGESGQGASQRFLEADVTFHELILRYCHNEMFAALIPSISAVLVGRTELGLQPDLPAHEALDNHDKLADALLNRDADAAETASRNILNEVRSALGTLN

SEQ ID NO: 14 - DNA, 43 bp, synthetic construct
  misc_feature 1..43: note = Primer sequence
  source 1..43: mol_type = other DNA
aatctcgtgatggcaggttgacgctgagaaggactacgattcc

SEQ ID NO: 15 - DNA, 21 bp, synthetic construct
  misc_feature 1..21: note = Primer sequence
  source 1..21: mol_type = other DNA
ccagcgaatgatggacttatc

SEQ ID NO: 16 - DNA, 45 bp, synthetic construct
  misc_feature 1..45: note = Primer sequence
  source 1..45: mol_type = other DNA
ataagtccatcattcgctgggccctcaatgacgaaggtcagcgtg

SEQ ID NO: 17 - DNA, 44 bp, synthetic construct
  misc_feature 1..44: note = Primer sequence
  source 1..44: mol_type = other DNA
cagttattggtgcccttcgacgttgaagctcttagcgatattgc

SEQ ID NO: 18 - DNA, 21 bp, synthetic construct
  misc_feature 1..21: note = Primer sequence
  source 1..21: mol_type = other DNA
tcgaagggcaccaataactgc

SEQ ID NO: 19 - DNA, 24 bp, synthetic construct
  misc_feature 1..24: note = Primer sequence
  source 1..24: mol_type = other DNA
cttttactttcaccagcgtttctg

SEQ ID NO: 20 - DNA, 24 bp, synthetic construct
  misc_feature 1..24: note = Primer sequence
  source 1..24: mol_type = other DNA
aacgctggtgaaagtaaaagatgc

SEQ ID NO: 21 - DNA, 45 bp, synthetic construct
  misc_feature 1..45: note = Primer sequence
  source 1..45: mol_type = other DNA
agctgtttcaaagcgcgcattgaattacactgtacctgttgcgtc

SEQ ID NO: 22 - DNA, 43 bp, synthetic construct
  misc_feature 1..43: note = Primer sequence
  source 1..43: mol_type = other DNA
atgcgcgctttgaaacagctgttttagagctagaaatagcaag

SEQ ID NO: 23 - DNA, 23 bp, synthetic construct
  misc_feature 1..23: note = Primer sequence
  source 1..23: mol_type = other DNA
caacctgccatcacgagattttc

SEQ ID NO: 24 - DNA, 21 bp, synthetic construct
  misc_feature 1..21: note = Primer sequence
  source 1..21: mol_type = other DNA
ttgaccgtgactacaccccac

SEQ ID NO: 25 - DNA, 21 bp, synthetic construct
  misc_feature 1..21: note = Primer sequence
  source 1..21: mol_type = other DNA
atcccatccccaccgaatctg